European Patent Application EP 4 417 695 A2, published August 21, 2024. Title: MODIFIED CIRCULAR RNAS AND METHODS OF USE THEREOF. Applicant: The Board of Trustees of the Leland Stanford Junior University. The sequence listing filed with the application follows.

SEQUENCE LISTING (20 sequences)

SEQ ID NO: 1 - DNA, 19 bp, synthetic construct
  misc_feature 1..19: note = qRT-PCR primer
  source 1..19: mol_type = other DNA
gaggcactcttccagcctt

SEQ ID NO: 2 - DNA, 20 bp, synthetic construct
  misc_feature 1..20: note = qRT-PCR primer
  source 1..20: mol_type = other DNA
aaggtagtttcgtggatgcc

SEQ ID NO: 3 - DNA, 20 bp, synthetic construct
  misc_feature 1..20: note = qRT-PCR primer
  source 1..20: mol_type = other DNA
tgtgggcaatgtcatcaaaa

SEQ ID NO: 4 - DNA, 21 bp, synthetic construct
  misc_feature 1..21: note = qRT-PCR primer
  source 1..21: mol_type = other DNA
gaagcacttgctacctcttgc

SEQ ID NO: 5 - DNA, 19 bp, synthetic construct
  misc_feature 1..19: note = qRT-PCR primer
  source 1..19: mol_type = other DNA
ggcaccatgggaagtgatt

SEQ ID NO: 6 - DNA, 20 bp, synthetic construct
  misc_feature 1..20: note = qRT-PCR primer
  source 1..20: mol_type = other DNA
atttggtaaggcctgagctg

SEQ ID NO: 7 - DNA, 21 bp, synthetic construct
  misc_feature 1..21: note = qRT-PCR primer
  source 1..21: mol_type = other DNA
gctcctaccctgtgtgtgtgt

SEQ ID NO: 8 - DNA, 21 bp, synthetic construct
  misc_feature 1..21: note = qRT-PCR primer
  source 1..21: mol_type = other DNA
tggtgagagtactgaggaaga

SEQ ID NO: 9 - DNA, 20 bp, synthetic construct
  misc_feature 1..20: note = qRT-PCR primer
  source 1..20: mol_type = other DNA
agggtacagatgggacatcg

SEQ ID NO: 10 - DNA, 20 bp, synthetic construct
  misc_feature 1..20: note = qRT-PCR primer
  source 1..20: mol_type = other DNA
aagggttcacgatgaggttg

SEQ ID NO: 11 - DNA, 21 bp, synthetic construct
  misc_feature 1..21: note = qRT-PCR primer
  source 1..21: mol_type = other DNA
tcttcatgtatgtgacactgc

SEQ ID NO: 12 - DNA, 18 bp, synthetic construct
  misc_feature 1..18: note = qRT-PCR primer
  source 1..18: mol_type = other DNA
cacacagtcaaggtcctt

SEQ ID NO: 13 - DNA, 25 bp, synthetic construct
  misc_feature 1..25: note = qRT-PCR primer
  source 1..25: mol_type = other DNA
gataagcttgccacctcagtagatg

SEQ ID NO: 14 - DNA, 22 bp, synthetic construct
  misc_feature 1..22: note = qRT-PCR primer
  source 1..22: mol_type = other DNA
atccatcacactggcatatgac

SEQ ID NO: 15 - DNA, 20 bp, synthetic construct
  misc_feature 1..20: note = qRT-PCR primer
  source 1..20: mol_type = other DNA
actacctgagcacccagtcc

SEQ ID NO: 16 - DNA, 20 bp, synthetic construct
  misc_feature 1..20: note = qRT-PCR primer
  source 1..20: mol_type = other DNA
cttgtacagctcgtccatgc

SEQ ID NO: 17-20 - skipped (4 entries)